European Patent Application EP 4 458 841 A1, published November 6, 2024. Title: Peptide having activities of skin condition improvement and uses thereof. Applicant: CAREGEN CO., LTD. The sequence listing filed with the application follows.

SEQUENCE LISTING (9 sequences)

SEQ ID NO: 1 - protein, 12 aa, Artificial Sequence
  Peptide 1
SHNFREEPEMRR

SEQ ID NO: 2 - DNA, 20 bp, Artificial Sequence
  Col1a1_F
caccctcaagagcctgagtc

SEQ ID NO: 3 - DNA, 20 bp, Artificial Sequence
  Col1a1_R
agacggctgagtagggaaca

SEQ ID NO: 4 - DNA, 20 bp, Artificial Sequence
  Fibronectin_F
ccaggaaccgagtacaccat

SEQ ID NO: 5 - DNA, 20 bp, Artificial Sequence
  Fibronectin_R
atacccaggttgggtgatga

SEQ ID NO: 6 - DNA, 20 bp, Artificial Sequence
  Elastin_F
gcaagacctggctttggact

SEQ ID NO: 7 - DNA, 21 bp, Artificial Sequence
  Elastin_R
gggagtttctggttagggctg

SEQ ID NO: 8 - DNA, 20 bp, Artificial Sequence
  GAPDH_F
ggagccaaaagggtcatcat

SEQ ID NO: 9 - DNA, 20 bp, Artificial Sequence
  GAPDH_R
gtgatggcatggactgtggt